European Patent Specification EP 3 544 967 B1, published June 28, 2023. Title: Salts of indazole derivative and crystals thereof. Applicant: Eisai R&D Management Co., Ltd. The sequence listing filed with the application follows.

SEQUENCE LISTING (8 sequences)

SEQ ID NO: 1 - DNA, 39 bp, artificial sequence
  mutagenesis primer
aagaacgtggtgcccctctctgacctgctgctggagatg

SEQ ID NO: 2 - DNA, 39 bp, artificial sequence
  mutagenesis primer
catctccagcagcaggtcagagaggggcaccacgttctt

SEQ ID NO: 3 - DNA, 39 bp, artificial sequence
  mutagenesis primer
aagaacgtggtgcccctcaatgacctgctgctggagatg

SEQ ID NO: 4 - DNA, 39 bp, artificial sequence
  mutagenesis primer
catctccagcagcaggtcattgaggggcaccacgttctt

SEQ ID NO: 5 - DNA, 39 bp, artificial sequence
  mutagenesis primer
aagaacgtggtgcccctctgtgacctgctgctggagatg

SEQ ID NO: 6 - DNA, 39 bp, artificial sequence
  mutagenesis primer
catctccagcagcaggtcacagaggggcaccacgttctt

SEQ ID NO: 7 - DNA, 39 bp, artificial sequence
  mutagenesis primer
aacgtggtgcccctctatggcctgctgctggagatgctg

SEQ ID NO: 8 - DNA, 39 bp, artificial sequence
  mutagenesis primer
cagcatctccagcagcaggccatagaggggcaccacgtt